European Patent Specification EP 3 445 859 B1, published January 21, 2026. Title: Elite Event EE-GH7 and methods and kits for identifying such event in biological samples. Applicant: Bayer CropScience NV Bayer CropScience LP. The sequence listing filed with the application follows.

SEQUENCE LISTING (13 sequences)

SEQ ID NO: 1 - DNA, 9328 bp, Artificial
  Sequence of the EE-GH7 transgenic locus
  misc_feature (1)..(1217): 5' flanking sequence
  misc_feature (1218)..(1219): RB (partial): partial right border region of the T-DNA of Agrobacterium tumefaciens
  misc_feature (1218)..(8032): Foreign DNA
  terminator (1277)..(1943): ThistonAt: histone terminator from Arabidopsis - complement
  misc_feature (1960)..(3036): hppdPf W336: mutated coding sequence of hppd - complement
  transit_peptide (3037)..(3408): TPotp Y-1Pa: transit peptide - complement
  promoter (3417)..(3929): Pcsvmv: promotor of the casein vein mosaic virus  - complement
  promoter (4028)..(4944): Ph4a748: histone promoter from Arabidopsis
  Intron (4984)..(5449): Intron1 h3At: first intron of gene II of histone H3
  transit_peptide (5463)..(5834): TPotpC: optimized transit peptide
  misc_feature (5835)..(7172): 2mepsps: double mutated EPSPsynhtase from corn
  terminator (7193)..(7859): ThistonAt: histone terminator from Arabidopsis
  misc_feature (8026)..(8032): LB (partial): partial left border region of the T-DNA of Agrobacterium tumefaciens
  misc_feature (8033)..(9328): 3' flanking sequence
ttcctaattctatcgtgcacatgtgatgcattcctttttttataacaaggaagttccaatttcatatctccaacgtagtatcatttagcataaaataaaagctagctaaaacttagcagttttggtcatttccatttagatatatatattttcaaaggtctatatttatctgtttgtattaataaaaaccatccattaaatggttgtaacgaattaaccaaaggaatctaaaacagtaaaaaaaagttttacctccattagtcagaagctgtttactcccctttcaagtcgtttcatcaaattaagaggttacatcaacaaatagggtgaatttttttactgttagtgacttcctcttttttttttttggtatcaggatgttgaatacattttttgtcagttactttctaaaatgataaataatttatcacgaaaaaacgtataagtcaaatattaatatatattttttaaaattattaataaaaaatataaatatcaaatactcataaataaatttttatttacaattgaattaaaatctgattgaaactcaaacaaatgcagcaaaaagtttgaaataatagtatagggatacgtaaaagttataaaacaaatacataaaatgtaaatatatggttttggatttggatttgaatttggatttggatttgggaatatttcttttcatgcggctggtgtctaatcgtgagattttctgacttgacggctaccattatttttccatccgcattatcttctttattgtactcaaaatatttcttatttgaaaatgaatttcttataaaatagtaaactaacattcggatttttaagccaatatcaatgttctattacattggaggaacatgggtcatgactcatgagcaccaatacacaattgtggtgtacatattgagccgtgtgacatatgcataaaattttactcattctccgttaatatcacacttttatcggtgtatataaattttattattttaatttatttttaaatttataatcatattaaaaataaaaaatattaaattaagtatttttttagagatattaaaattaaaaatagttttaaaatttatatttatatacaaatgtgtttataattgaaatctatatgacgtgcacataattattattatcaaactccgaatagttccatcaattttatcatttatgtatttggaagccttgaaacagaacaacagtactgggccccctcgagggcgatcgctacgtacctgcaggcccgggttaattaaggcccgatcaaatctgagggacgttaaagcgatgataaattggaaccagaatatagaatctttgttctgctctagcttttcttctgtacattttttacgattagactatgattttcattcaataaccaaaattctgaagtttgtcatcaagttgctcaatcaaacttgtaccggtttgtttcggttttatatcagctcactgttacactttaaccaaaatcggtttatgtcttaataaaggaattgagtcggtttaactcatatccgtaccaatgcgacgtcgtgtccgcgtttcagtagctttgctcattgtcttctacgggaactttcccggacataggaaccgccctttcgttatcctcatccatcgtgaaatcaggaaataaatgttcgaagatttgaggtcaaaagtcgaatttcatgttgtctcttctatttagatacaaaattgaagcaattttcaccaatttaatgccaaaatttaaaacaacgctgataaagtgaaacttgattcgatttatatttcaaccgaaactgctgaagcaagaagaaaaagcgtaattacacataacaagaacgctaccgcaaactactaaacgccaaacccaatacaaaagtaaaacgcagacgcttaagtgagaaacccagaaaacacaaacgcggatcgggcgacgcgtgctagcttttaatcagcggtcaaaacccctctacgaacttgatccctctctatcgattcgaaaagtgctttgaagttccattctccgaagccatcgtcccctttacgctgaatgaactcaaagaaaacgggtcccatgagagtctcggaaaagatttgtaacaggagcctcttatcaccctcaaccgaagaaccatcgagaagtatacccctggcttgcagttggtccacgggttccccatgatcaggcaggcgtccttctagcatctcatagtaagtatcgggaggtgcagtcatgaatctcatacctatcttcttcaatgcatcccaggttttcacaagatcatcagtcagaaaagcgacatgctgaatgccttcaccattgaactgcataagaaactcttcgatttgtcctgcacctttgcttgactcttcgttgagtggaatccttatcataccatctggagcgctcatagcctttgatgtgagaccagtatactctcctttgatgtcaaagtatctagcttccctaaagttgaagagtttctcatagaagttagcccagtataccattcgtccacgatagacgttgtgtgtcaaatgatcaataaccttcaagccagcaccgacaggatttcgttccacgccttcaagatagacgaaatctatgtcgtagatagaactgccctctccgaatctgtcgataagatacaacggtgcaccaccgatgcctttgatggctggaagattcaattccataggtccagtgtcaatgtgaataggctgagctccaagttctaatgccctattgtaggctttctgggaatccttaactcgaaatgccatgccacaaacggatggtccatgttcggcagcaaagtagcttgctatagagttaggttcgttgttcaagatcaggttaatctctccttgccgatataggtgcacgttcttactgcgatgtgtagctaccttagtaaaccccataatctcaaagatgggttcaagggtcccaggtgtaggagaagcaaactcaatgaactcgaaacccatgagtcccataggattctcgtatagatcagccatgcatctaatcctacctccgttgctaacattccccagcgatctggaagatctccgagcaactggcaaactagcagtactcttcaacccttgaaatggtgccacagctgtggcagagctggccatcatcacagtgggagccatagatagcggaggtaagtaggataaggtctcaaacttcttgttgccataggctggccagacttgcatatactgtactctcccaccgttgctcggaagtgttgagaagtcattagccttcttagtggttggaaatgcagcatttgacttaagacctgtgaacggagccaccatattagcttgggctggtgcggtacgtgaaacagtggcaactgaagatgaaatactagccatggttttggacaaacttacaaatttctctgaagttgtatcctcagtacttcaaagaaaatagcttacaccaaattttttcttgttttcacaaatgccgaacttggttccttatataggaaaactcaagggcaaaaatgacacggaaaaatataaaaggataagtagtgggggataagattcctttgtgataaggttactttccgcccttacattttccaccttacatgtgtcctctatgtctctttcacaatcaccgaccttatcttcttcttttcattgttgtcgtcagtgcttacgtcttcaagattcttttcttcgcctggttcttctttttcaatttctacgtattcttcttcgtattctggcagtataggatcttgtatctgtacattcttcatttttgaacataggttgcatatgtgccgcatattgatctgcttcttgctgagctcacataatacttccatagtttttcccgtaaacattggattcttgatgctacatcttggataattaccttcgcggccgcttggcgcgccgaattcgatatcattaccctgttatccctaaagcttattaatataacttcgtatagcatacattatacgaagttatgtttgtcgaggagaaatatgagtcgaggcatggatacactaagttcccctgaagtgagcatgatctttgatgctgagatgattcccagagcaagatagtttgtgctgcaagtgacacaattgtaatgaaaccaccactcaacgaatttacttgtggctttgacatgtcgtgtgctctgtttgtatttgtgagtgccggttggtaattatttttgttaatgtgattttaaaacctcttatgtaaatagttactttatctattgaagtgtgttcttgtggtctatagtttctcaaagggaaattaaaatgttgacatcccatttacaattgataacttggtatacacaaactttgtaaatttggtgatatttatggtcgaaagaaggcaatacccattgtatgttccaatatcaatatcaatacgataacttgataatactaacatatgattgtcattgtttttccagtatcaatatacattaagctactacaaaattagtataaatcactatattataaatctttttcggttgtaacttgtaattcgtgggtttttaaaataaaagcatgtgaaaattttcaaataatgtgatggcgcaattttattttccgagttccaaaatattgccgcttcattaccctaatttgtggcgccacatgtaaaacaaaagacgattcttagtggctatcactgccatcacgcggatcactaatatgaaccgtcgattaaaacagatcgacggtttatacatcattttattgtacacacggatcgatatctcagccgttagatttaatatgcgatctgattgctcaaaaaatagactctccgtctttgcctataaaaacaatttcacatctttctcacccaaatctactcttaaccgttcttcttcttctacagacatcaatttctctcgactctagaggatccaagcttatcgatttcgaacccctcaggcgaagaacaggtatgatttgtttgtaattagatcaggggtttaggtctttccattactttttaatgttttttctgttactgtctccgcgatctgattttacgacaatagagtttcgggttttgtcccattccagtttgaaaataaaggtccgtcttttaagtttgctggatcgataaacctgtgaagattgagtctagtcgatttattggatgatccattcttcatcgtttttttcttgcttcgaagttctgtataaccagatttgtctgtgtgcgattgtcattacctagccgtgtatcgagaactagggttttcgagtcaattttgccccttttggttatatctggttcgataacgattcatctggattagggttttaagtggtgacgtttagtattccaatttcttcaaaatttagttatggataatgaaaatccccaattgactgttcaatttcttgttaaatgcgcagatcacaatggcttcgatctcctcctcagtcgcgaccgttagccggaccgcccctgctcaggccaacatggtggctccgttcaccggccttaagtccaacgccgccttccccaccaccaagaaggctaacgacttctccacccttcccagcaacggtggaagagttcaatgtatgcaggtgtggccggcctacggcaacaagaagttcgagacgctgtcgtacctgccgccgctgtctatggcgcccaccgtgatgatggcctcgtcggccaccgccgtcgctccgttccaggggctcaagtccaccgccagcctccccgtcgcccgccgctcctccagaagcctcggcaacgtcagcaacggcggaaggatccggtgcatggccggcgccgaggagatcgtgctgcagcccatcaaggagatctccggcaccgtcaagctgccggggtccaagtcgctttccaaccggatcctcctactcgccgccctgtccgaggggacaacagtggttgataacctgctgaacagtgaggatgtccactacatgctcggggccttgaggactcttggtctctctgtcgaagcggacaaagctgccaaaagagctgtagttgttggctgtggtggaaagttcccagttgaggatgctaaagaggaagtgcagctcttcttggggaatgctggaatcgcaatgcggtccttgacagcagctgttactgctgctggtggaaatgcaacttacgtgcttgatggagtaccaagaatgagggagagacccattggcgacttggttgtcggattgaagcagcttggtgcagatgttgattgtttccttggcactgactgcccacctgttcgtgtcaatggaatcggagggctacctggtggcaaggtcaagctgtctggctccatcagcagtcagtacttgagtgccttgctgatggctgctcctttggctcttggggatgtggagattgaaatcattgataaattaatctccattccgtacgtcgaaatgacattgagattgatggagcgttttggtgtgaaagcagagcattctgatagctgggacagattctacattaagggaggtcaaaaatacaagtcccctaaaaatgcctatgttgaaggtgatgcctcaagcgcaagctatttcttggctggtgctgcaattactggagggactgtgactgtggaaggttgtggcaccaccagtttgcagggtgatgtgaagtttgctgaggtactggagatgatgggagcgaaggttacatggaccgagactagcgtaactgttactggcccaccgcgggagccatttgggaggaaacacctcaaggcgattgatgtcaacatgaacaagatgcctgatgtcgccatgactcttgctgtggttgccctctttgccgatggcccgacagccatcagagacgtggcttcctggagagtaaaggagaccgagaggatggttgcgatccggacggagctaaccaagctgggagcatctgttgaggaagggccggactactgcatcatcacgccgccggagaagctgaacgtgacggcgatcgacacgtacgacgaccacaggatggcgatggctttctcccttgccgcctgtgccgaggtccccgtcaccatccgggaccctgggtgcacccggaagaccttccccgactacttcgatgtgctgagcactttcgtcaagaattaagctctagaactagtggatcccccgatccgcgtttgtgttttctgggtttctcacttaagcgtctgcgttttacttttgtattgggtttggcgtttagtagtttgcggtagcgttcttgttatgtgtaattacgctttttcttcttgcttcagcagtttcggttgaaatataaatcgaatcaagtttcactttatcagcgttgttttaaattttggcattaaattggtgaaaattgcttcaattttgtatctaaatagaagagacaacatgaaattcgacttttgacctcaaatcttcgaacatttatttcctgatttcacgatggatgaggataacgaaagggcggttcctatgtccgggaaagttcccgtagaagacaatgagcaaagctactgaaacgcggacacgacgtcgcattggtacggatatgagttaaaccgactcaattcctttattaagacataaaccgattttggttaaagtgtaacagtgagctgatataaaaccgaaacaaaccggtacaagtttgattgagcaacttgatgacaaacttcagaattttggttattgaatgaaaatcatagtctaatcgtaaaaaatgtacagaagaaaagctagagcagaacaaagattctatattctggttccaatttatcatcgctttaacgtccctcagatttgatcgggaaacataacttcgtatagcatacattatacgaagttatcaaaacgtcgtgagacagtttggttaactataacggtcctaaggtagcgatcgaggcattacggcattacggcactcgcgagggtccgaatctatgtcgggtgcggagaaagaggtaatgaaatggcaatttacaatagaagatagaattgatgcaatcagttttagaataaaaacgatatgtcgatcgtgtaaattttgaaaatattgactgaatggtttcgattaaacctaactttcaagtttcaatcataagatgtttatcccctaaaagattcctagttgctaagagtttacaaaatagagctatccattcgaattagacttattcaaatagtttaaattagtggtctaatgtcgaaggtatgctcgaaagttttgaagaaaaatattaaatttaaaaattgagttttgtacaaaaatttaattatttttttatttaaataagatttgagctcaaatttcaatatttaaagtccgagctttactcaatttagtctagtacgctcttaaaggtataacataatttaatctattttatatatatgaaaaatggaaatcgacagatccatgattatttattactaaggaccccatttaagttcccaggacaatgaagggacatcaactattaataaataaatggaatggtaagtgtcatcagcatagtgcgcatctagacaagctcttgacgatatataaatgtatatgtcacttaacaaccgtgcaaaccttatctgattaaaccaaggcaaaacgcccaaccagattaattaaggggcatatatagcacagatcagacgtgaccagtcagggattagggggtgagctcacctcaccacaaatgcctttcattttggctcgacaatctttataatctgtccatgcaaaaggatgcattccaggtcaataaaatgtagtcactgagttgtagagatcaaaccatttgtctccaagaacatacatgagtggactttgagcctcaaactttgttatatttgtgtggttaggtataaataataatcttcctcactcttctcaattatttggcaactgtagaaataattgccaaaaagctttgaaagttttgtcaattttgttacattgtgtcaattcaccttttgaaggtgcaagaacttgtctcaaaattgagtctttacatatatattataatgatttctgaaagtttttaacatgagcagtacaagtattattggtactaattactcataattttgtttttgtttttgtggtgaaaatggtcgtgaaagaggctttcttttaagaatcaagatttgagaaagtattcttttgttttgttttgttttattggcaaaccaatgattagatatgttaatagaatttaacttatagacacgtttaggacataacttttaacattgtccttaaaaagttttaaaagtctaattaa

SEQ ID NO: 2 - DNA, 2526 bp, Artificial
  EE-GH7 insertion locus
  misc_feature (1)..(1217): 5' flanking sequence
  misc_feature (1218)..(1230): TSD: Target site deletion
  misc_feature (1231)..(2526): 3' flanking sequence
ttcctaattctatcgtgcacatgtgatgcattcctttttttataacaaggaagttccaatttcatatctccaacgtagtatcatttagcataaaataaaagctagctaaaacttagcagttttggtcatttccatttagatatatatattttcaaaggtctatatttatctgtttgtattaataaaaaccatccattaaatggttgtaacgaattaaccaaaggaatctaaaacagtaaaaaaaagttttacctccattagtcagaagctgtttactcccctttcaagtcgtttcatcaaattaagaggttacatcaacaaatagggtgaatttttttactgttagtgacttcctcttttttttttttggtatcaggatgttgaatacattttttgtcagttactttctaaaatgataaataatttatcacgaaaaaacgtataagtcaaatattaatatatattttttaaaattattaataaaaaatataaatatcaaatactcataaataaatttttatttacaattgaattaaaatctgattgaaactcaaacaaatgcagcaaaaagtttgaaataatagtatagggatacgtaaaagttataaaacaaatacataaaatgtaaatatatggttttggatttggatttgaatttggatttggatttgggaatatttcttttcatgcggctggtgtctaatcgtgagattttctgacttgacggctaccattatttttccatccgcattatcttctttattgtactcaaaatatttcttatttgaaaatgaatttcttataaaatagtaaactaacattcggatttttaagccaatatcaatgttctattacattggaggaacatgggtcatgactcatgagcaccaatacacaattgtggtgtacatattgagccgtgtgacatatgcataaaattttactcattctccgttaatatcacacttttatcggtgtatataaattttattattttaatttatttttaaatttataatcatattaaaaataaaaaatattaaattaagtatttttttagagatattaaaattaaaaatagttttaaaatttatatttatatacaaatgtgtttataattgaaatctatatgacgtgcacataattattattatcaaactccgaatagttccatcaattttatcatttatgtatttggaagccttgaaacagaacaatgcttaagtaagcatagaagatagaattgatgcaatcagttttagaataaaaacgatatgtcgatcgtgtaaattttgaaaatattgactgaatggtttcgattaaacctaactttcaagtttcaatcataagatgtttatcccctaaaagattcctagttgctaagagtttacaaaatagagctatccattcgaattagacttattcaaatagtttaaattagtggtctaatgtcgaaggtatgctcgaaagttttgaagaaaaatattaaatttaaaaattgagttttgtacaaaaatttaattatttttttatttaaataagatttgagctcaaatttcaatatttaaagtccgagctttactcaatttagtctagtacgctcttaaaggtataacataatttaatctattttatatatatgaaaaatggaaatcgacagatccatgattatttattactaaggaccccatttaagttcccaggacaatgaagggacatcaactattaataaataaatggaatggtaagtgtcatcagcatagtgcgcatctagacaagctcttgacgatatataaatgtatatgtcacttaacaaccgtgcaaaccttatctgattaaaccaaggcaaaacgcccaaccagattaattaaggggcatatatagcacagatcagacgtgaccagtcagggattagggggtgagctcacctcaccacaaatgcctttcattttggctcgacaatctttataatctgtccatgcaaaaggatgcattccaggtcaataaaatgtagtcactgagttgtagagatcaaaccatttgtctccaagaacatacatgagtggactttgagcctcaaactttgttatatttgtgtggttaggtataaataataatcttcctcactcttctcaattatttggcaactgtagaaataattgccaaaaagctttgaaagttttgtcaattttgttacattgtgtcaattcaccttttgaaggtgcaagaacttgtctcaaaattgagtctttacatatatattataatgatttctgaaagtttttaacatgagcagtacaagtattattggtactaattactcataattttgtttttgtttttgtggtgaaaatggtcgtgaaagaggctttcttttaagaatcaagatttgagaaagtattcttttgttttgttttgttttattggcaaaccaatgattagatatgttaatagaatttaacttatagacacgtttaggacataacttttaacattgtccttaaaaagttttaaaagtctaattaa

SEQ ID NO: 3 - DNA, 27 bp, Artificial
  primer PRIM0728
ctccgaatagttccatcaattttatca

SEQ ID NO: 4 - DNA, 21 bp, Artificial
  Primer PRIM0643
tgatcgggccttaattaaccc

SEQ ID NO: 5 - DNA, 30 bp, artificial
  primer PRIM0638
cgaatagttccatcaattttatcatttatg

SEQ ID NO: 6 - DNA, 19 bp, artificial
  primer PRIM0639
tcgggccttaattaacccg

SEQ ID NO: 7 - DNA, 18 bp, artificial
  probe TM1576
agaacaacagtactgggc

SEQ ID NO: 8 - DNA, 23 bp, artificial
  Primer KVM157
cacatgacttagcccatctttgc

SEQ ID NO: 9 - DNA, 21 bp, artificial
  Primer KVM158
cccacccttttttggtttagc

SEQ ID NO: 10 - DNA, 26 bp, artificial
  Primer TM1304
tgcaggttttggtgccactgtgaatg

SEQ ID NO: 11 - DNA, 26 bp, artificial
  Primer PRIM0726
caaactccgaatagttccatcaattt

SEQ ID NO: 12 - DNA, 49 bp, artificial
  Primer PRIM0733
gaaggtcggagtcaacggattgcttacttaagcattgttctgtttcaag

SEQ ID NO: 13 - DNA, 45 bp, artificial
  Primer PRIM0731
gaaggtgaccaagttcatgctggcccagtactgttgttctgtttc